European Patent Application EP 4 310 102 A1, published January 24, 2024. Title: PEPTIDE COMBINATION, CHIMERIC PEPTIDE, IMMUNOGENIC COMPOSITION, USE OF THE PEPTIDE COMBINATION, USE OF THE CHIMERIC PEPTIDE, USE OF A COMPOSITION, METHOD TO INDUCE IMMUNE RESPONSE AND KIT. Applicant: EMBRAPA-EMPRESA BRASILEIRA DE PESQUISA AGROPECUARIA. Application BR 10 2021 004904 9. The sequence listing filed with the application follows.

SEQUENCE LISTING (12 sequences)

SEQ ID NO: 1 - protein, 30 aa, Rhipicephalus microplus
  PEPTIDE (1)..(11): 73% identity with "insect cuticle protein" of I. scapularis
  PEPTIDE (12)..(16): Linker
  PEPTIDE (17)..(30): peptide epitope of Clostridium tetani tetanus toxin
TNEPGTAPGETGPGPGQYIKANSKFIGITE

SEQ ID NO: 2 - protein, 48 aa, Rhipicephalus microplus
  PEPTIDE (1)..(12): 67% identity with "insect cuticle protein" of I. scapularis.
  PEPTIDE (13)..(17): Linker
  PEPTIDE (18)..(34): 67% identity with "insect cuticle protein" of I. scapularis.
  PEPTIDE (35)..(39): Linker
  PEPTIDE (40)..(48): 67% identity with "insect cuticle protein" of I. scapularis.
VAPTANPSPAPWGPGPGQSPVAPGAYNPPAPATYGPGPGNQSPQPQPA

SEQ ID NO: 3 - protein, 29 aa, Rhipicephalus microplus
  PEPTIDE (1)..(29): 88% identity with "Chitin binding protein/embryo" of I. scapularis.
PASVTPPPPRQTASGPGPGGPPSSQTPRA

SEQ ID NO: 4 - protein, 19 aa, Rhipicephalus microplus
  PEPTIDE (1)..(19): 70% identity with "Embryonated eggs protein" of I. scapularis.
ATQQGNEGQQGSSDKGQEL

SEQ ID NO: 5 - protein, 12 aa, Rhipicephalus microplus
  PEPTIDE (1)..(12): 55% identity with "Embryonated eggs protein" of I. scapularis.
AVDPSSPEQHPE

SEQ ID NO: 6 - protein, 22 aa, Rhipicephalus microplus
  PEPTIDE (1)..(21): 90% identity with "TPR Repetition (Signal transduction mechanisms)" of I. scapularis
VGGDGPAPAKHRSGDSGEGVDD

SEQ ID NO: 7 - protein, 33 aa, Rhipicephalus microplus
  PEPTIDE (1)..(14): 30% identity with "Zinc-dependent metalloprotease" of R. microplus
  PEPTIDE (15)..(19): Linker
  PEPTIDE (20)..(33): peptide epitope of Clostridium tetani tetanus toxin
EDHGRRTEDPEPDCGPGPGQYIKANSKFIGITE

SEQ ID NO: 8 - protein, 20 aa, Rhipicephalus microplus
  PEPTIDE (1)..(20): 45% identity with "Kazal-type serine protease inhibitor proteins" of I. scapularis.
PVEDEDKDSQETQEPGGPWS

SEQ ID NO: 9 - protein, 16 aa, Rhipicephalus microplus
  PEPTIDE (1)..(16): 67% identity with  "Insect cuticle protein - chitin bond" of I. scapularis.
TNEPGTAPGATGDAQY

SEQ ID NO: 10 - protein, 21 aa, Rhipicephalus microplus
  PEPTIDE (1)..(21): 43% identity with "Kunitz / Trypsin inhibitor domain" of R. microplus.
FPPYQGRPGATNEWPGSPYSP

SEQ ID NO: 11 - protein, 24 aa, Rhipicephalus microplus
  PEPTIDE (1)..(24): 43% identity with "trypsin inhibitor(BPTI) Kunitz" of R. microplus.
TKPSPPSQEAPSSTDEGWYPPRRR

SEQ ID NO: 12 - protein, 12 aa, Rhipicephalus microplus
  PEPTIDE (1)..(10): 35% identity with "Saliva molecules that modulate host response" of I. scapularis.
DFDDSPSDEHTG